European Patent Application EP 4 455 298 A1, published October 30, 2024. Title: 遺伝子導入率予測方法. Applicant: 武田薬品工業株式会社. The sequence listing filed with the application follows.

SEQUENCE LISTING (3 sequences)

SEQ ID NO: 1 - DNA, 2652 bp, Homo sapiens
  source 1..2652: mol_type = other DNA
atggactggacctggaggatcctgtttctggtggccgccgccacaggagcccacagccaggtgcagctgcagcagagcggacctggcctggtgacacccagccagaccctgagcctgacctgtgccatctccggcgatagcgtgagcagcaacagcgccacctggaactggatcaggcagagccccagcagaggactggagtggctgggcaggacctactacaggagcaagtggtacaacgactacgccgtgagcgtgaagagcaggatgagcatcaaccccgacaccagcaagaaccagttctccctgcagctgaactccgtgacccccgaggacaccgccgtgtactactgcgccaggggcatgatgacctactactacggcatggacgtgtggggccagggaaccaccgtgaccgtgagcagcggcatcctgggcagcggcggcggcggcagcggcggcggcggcagcggaggaggcggaagccagcctgtgctgacccagagcagcagcctgagcgctagccctggagctagcgccagcctgacctgcaccctgagaagcggcatcaacgtgggcccctacaggatctactggtaccagcagaagcctggcagccccccccagtacctgctgaactacaagagcgacagcgacaagcagcagggcagcggcgtgcctagcagattcagcggcagcaaggatgccagcgccaacgccggagtgctgctgatcagcggcctgaggagcgaggatgaggccgactactactgcatgatctggcacagcagcgccgccgtgtttggaggcggaacccagctgaccgtgctgagcgcggccgcaaccaccacccccgcccctagacctcctacacccgctcccacaatcgccagccagcctctgtctttaagacccgaggcttgtagacccgctgctggcggcgccgtgcataccagaggactggacttcgcttgtgacatctacatctgggctcctttagccggcacatgtggagtgctgctgctgtctttagtgatcactttatactgcaagaggggtcgtaagaagctgctgtacatcttcaagcagcccttcatgaggcccgtgcagaccacccaagaagaggacggctgcagctgtcgttttcccgaagaggaggagggcggctgcgagctgagggtgaagttcagcagaagcgccgatgcccccgcttaccagcaaggtcagaaccagctgtacaacgagctgaatttaggtcgtagggaggagtacgacgtgctggacaagaggaggggcagagaccccgaaatgggcggcaagcctcgtaggaagaacccccaagaaggtttatacaacgagctgcagaaggacaagatggccgaggcctacagcgagatcggcatgaagggcgagaggaggagaggcaagggccacgacggtttataccaaggtctgagcaccgccaccaaggacacctacgatgctttacacatgcaagctttacctcctcgtggaagcggagctactaacttcagcctgctgaagcaggctggagacgtggaggagaaccctggacccatgcttctcctggtgacaagccttctgctctgtgagttaccacacccagcattcctcctgatcccacgcaaagtgtgtaacggaataggtattggtgaatttaaagactcactctccataaatgctacgaatattaaacacttcaaaaactgcacctccatcagtggcgatctccacatcctgccggtggcatttaggggtgactccttcacacatactcctcctctggacccacaggaactggatattctgaaaaccgtaaaggaaatcacagggtttttgctgattcaggcttggcctgaaaacaggacggacctccatgcctttgagaacctagaaatcatacgcggcaggaccaagcaacatggtcagttttctcttgcagtcgtcagcctgaacataacatccttgggattacgctccctcaaggagataagtgatggagatgtgataatttcaggaaacaaaaatttgtgctatgcaaatacaataaactggaaaaaactgtttgggacctccggtcagaaaaccaaaattataagcaacagaggtgaaaacagctgcaaggccacaggccaggtctgccatgccttgtgctcccccgagggctgctggggcccggagcccagggactgcgtctcttgccggaatgtcagccgaggcagggaatgcgtggacaagtgcaaccttctggagggtgagccaagggagtttgtggagaactctgagtgcatacagtgccacccagagtgcctgcctcaggccatgaacatcacctgcacaggacggggaccagacaactgtatccagtgtgcccactacattgacggcccccactgcgtcaagacctgcccggcaggagtcatgggagaaaacaacaccctggtctggaagtacgcagacgccggccatgtgtgccacctgtgccatccaaactgcacctacggatgcactgggccaggtcttgaaggctgtcccacgaatgggcctaagatcccgtccatcgccactgggatggtgggggccctcctcttgctgctggtggtggccctggggatcggcctcttcatgtaa

SEQ ID NO: 2 - DNA, 2472 bp, Homo sapiens
  source 1..2472: mol_type = other DNA
atggactggacctggaggatcctgtttctggtggccgccgccacaggagcccacagccaggtgcagctgcagcagagcggacctggcctggtgacacccagccagaccctgagcctgacctgtgccatctccggcgatagcgtgagcagcaacagcgccacctggaactggatcaggcagagccccagcagaggactggagtggctgggcaggacctactacaggagcaagtggtacaacgactacgccgtgagcgtgaagagcaggatgagcatcaaccccgacaccagcaagaaccagttctccctgcagctgaactccgtgacccccgaggacaccgccgtgtactactgcgccaggggcatgatgacctactactacggcatggacgtgtggggccagggaaccaccgtgaccgtgagcagcggcatcctgggcagcggcggcggcggcagcggcggcggcggcagcggaggaggcggaagccagcctgtgctgacccagagcagcagcctgagcgctagccctggagctagcgccagcctgacctgcaccctgagaagcggcatcaacgtgggcccctacaggatctactggtaccagcagaagcctggcagccccccccagtacctgctgaactacaagagcgacagcgacaagcagcagggcagcggcgtgcctagcagattcagcggcagcaaggatgccagcgccaacgccggagtgctgctgatcagcggcctgaggagcgaggatgaggccgactactactgcatgatctggcacagcagcgccgccgtgtttggaggcggaacccagctgaccgtgctgagcgcggccgcaaccaccacccccgcccctagacctcctacacccgctcccacaatcgccagccagcctctgtctttaagacccgaggcttgtagacccgctgctggcggcgccgtgcataccagaggactggacttcgcttgtgacatctacatctgggctcctttagccggcacatgtggagtgctgctgctgtctttagtgatcactttatactgcaagaggggtcgtaagaagctgctgtacatcttcaagcagcccttcatgaggcccgtgcagaccacccaagaagaggacggctgcagctgtcgttttcccgaagaggaggagggcggctgcgagctgagggtgaagttcagcagaagcgccgatgcccccgcttaccagcaaggtcagaaccagctgtacaacgagctgaatttaggtcgtagggaggagtacgacgtgctggacaagaggaggggcagagaccccgaaatgggcggcaagcctcgtaggaagaacccccaagaaggtttatacaacgagctgcagaaggacaagatggccgaggcctacagcgagatcggcatgaagggcgagaggaggagaggcaagggccacgacggtttataccaaggtctgagcaccgccaccaaggacacctacgatgctttacacatgcaagctttacctcctcgtggaagcggagctactaacttcagcctgctgaagcaggctggagacgtggaggagaaccctggaccctgcatgttccatgtgagcttcaggtacatcttcggactgcctcctctcatcctggtcctcctccccgtggccagctccgactgtgacatcgaaggaaaggatggcaagcagtacgaaagcgtgctgatggtgagcatcgatcagctcctggattccatgaaggaaatcggctccaactgcctcaacaatgagttcaacttttttaagaggcatatctgcgacgccaacaaggagggcatgtttctgttcagggccgccaggaagctgagacagttcctcaagatgaatagcaccggcgacttcgacctccatctgctgaaggtgtccgagggaaccaccatcctgctgaactgcaccggccaagtgaagggaagaaaacctgctgccctgggcgaggctcagcctaccaagagcctggaggagaacaaaagcctgaaggagcagaagaagctgaacgacctgtgcttcctcaagaggctcctgcaggagattaagacctgttggaacaagatcctgatgggcacaaaggagcacggcagcggcgccaccaacttctctctgctgaagcaagccggcgatgtggaggagaatcccggccccatggctctgctgctcgccctgagcctgctcgtcctctggacctcccctgctcctaccctgagcggcaccaatgacgctgaagactgctgcctgtccgtgacccagaagcctatccccggatatatcgtgaggaattttcattacctcctgatcaaggacggctgtagagtgcccgccgtcgtgttcacaacactcagaggcaggcagctgtgtgctccccccgaccagccttgggtggagagaatcattcagagactgcaaaggacctccgctaagatgaagaggaggtccagc

SEQ ID NO: 3 - DNA, 711 bp, synthetic construct
  source 1..711: mol_type = other DNA
atggtgagcaagggcgaggaggataacatggccatcatcaaggagttcatgcgcttcaaggtgcacatggagggctccgtgaacggccacgagttcgagatcgagggcgagggcgagggccgcccctacgagggcacccagaccgccaagctgaaggtgaccaagggtggccccctgcccttcgcctgggacatcctgtcccctcagttcatgtacggctccaaggcctacgtgaagcaccccgccgacatccccgactacttgaagctgtccttccccgagggcttcaagtgggagcgcgtgatgaacttcgaggacggcggcgtggtgaccgtgacccaggactcctccctgcaggacggcgagttcatctacaaggtgaagctgcgcggcaccaacttcccctccgacggccccgtaatgcagaagaagaccatgggctgggaggcctcctccgagcggatgtaccccgaggacggcgccctgaagggcgagatcaagcagaggctgaagctgaaggacggcggccactacgacgctgaggtcaagaccacctacaaggccaagaagcccgtgcagctgcccggcgcctacaacgtcaacatcaagttggacatcacctcccacaacgaggactacaccatcgtggaacagtacgaacgcgccgagggccgccactccaccggcggcatggacgagctgtacaagtga